European Patent Specification EP 3 964 578 B1, published May 13, 2026. Title: METHYLATION-BASED MODIFIED TUMOR MARKER STAMP-EP8 AND APPLICATION THEREOF. Applicant: SHANGHAI EPIPROBE BIOTECHNOLOGY CO.,LTD. The sequence listing filed with the application follows.

SEQUENCE LISTING (18 sequences)

SEQ ID NO: 1 - DNA, 2700 bp, Homo sapiens
cggatcgctaccgcggccttgggctcagttcctggagccggcctcgggtccggcctcgggtccctcctcggcggcgtccactgctgccgcagaagagacgctcccaggatttggtttccagtgggagaaggaaggcgccgcaaataccatcggctgcgaggcgactgtggtggtcgaaggaacgtgatcctttgtcagctcagcggagccgaagtgatcgccgagttggctgagcagcgccgagggagtttagaatccgctgcagaaaacctaccagcttcttcgcggacacagcaggtaatgttcttaggcttctggagttagtgagtagccggcctgcaggccggtaaataactccgatctagccccttggtttatttctttcgttcgcgccttgaatggaggcgccatggcacagtctggcagaggaggcctgccctggcgggcgctactcagggcccctgcgttgagaatgccgagtgaggtgctgaggtttggagagaaaaaggtggcgttttcatcccttggaatatcgggcctctccagctgaagcctccggatcgacacaacacaactcccggatcgacgcaacacaactccccgccagccccttcccttccagcgggctggacacaggtgcgtgggcctcgcagcccggcgcgcacggttgcgcctttggatacctgcgacaggactcggccagaaccgtgtcccagggcagagaaaaccctggcaacctttaacgttctccctgacgcggagaatcctgcgccaacggggccttccacttcgggagactcaatcgccacccggtccccaactttcgtcttccagaagaaaaatccatgaggaggaatgggggggtcccccgaccagaccagcaagaaagggcccagttaggagtgacctcagcgccacgagggttccactgctttgatggccacacgcttttgcaaacggtttgggggtggagagacaccaggtgatggtagggaagggcggtggtgactggcacggctaagacactgcggagggtttcgctgtggagatgagaaggtggaggttctgggcactgtggctgcgagtgtgagcgatgcgtttgtgggaatcagaggagcggatttgggaaaagtgaatccttgagattcagggccttactttcgttaggggtgtgtgaagcacactgggtgtcaggagaggatgggaatgggattcgagaggcctttttttggactcctcgagagaaaatggagagagtctcgaacccaggagataggaggcgtattttccccatgcacccatggatcacgcccccgcccccacattccccccgtaggaggcaagacctgagcgcttactcacgtggctcccccatccgttccgcgtccatctccaagactgcctcacagggacccccaggaggctccgaaccatccagctttctgtcaccgccgccgccaccagcgttgtgaacctctgaccctcgcggctctgcgtccattctcaggtactgaaagttttccgggctcttccgcacccgcggatgtggcgaagccgcggggcagctccgctcgcgctccagtcgcaggatgtccttgaccgagaagggggtggaggtgacggggctcagcagcatcccgaaggcggatggggcggggccgaggaggtccgggtgaggagcggcaccctgaacttcccgtcttgtcgctgcaggccccgcagacagacccaagctctgggacagacgcccagcgtcccagacagcgccttcctctgggccatgctggtaggcccgggtccagggccgggtgacgagaccgtagccccccattggttctcgcagaaaccacgtgctagctctgcaccttcctcccccagcgctttcttcccgcgcccgtcgaatcctctccagtccccagtcgccttcctgggaggtttggttcgtattgacggttctcaaagcaaagaaaacgtggagagacagtgctgcgcgcggcttggatctccgtcaatacggtactagcgggagcttccgaggtcaacctagggtccacggggaccctcctagtggacatgcggggattggaggtggagtccttgctgtgcaacccgatccggtccatccagcctggtcttagctcaactctgcattcttatggcggaggaaagctaagatagagacagctgggacccgcggaatttgaggcgcgcgctgggatcttacgtgcgcagaggccggaccgcagagtagaagtgagtcttgacccaccagggcctatattgagatggaaacctctctctttgaacagaatccaggtctgcggagtcccgacccgccacttcctaggagcagcttctcagccccaggaccgaggaatgggtgtgggggctacatgtggggagccctcgacctcttaaagggctccgcgaatggtgggggagactggaaggcaatctctgcggcccgcgcaaagtggtcagaggcgggagtgggggtgggggggggtgggcttccgtcgcccttggcgtccccacgttctttttcttcctctcctttatcctccttaaagcggattgcctggagcgtgccagcttgtgtgcgcgtataaatgcggcgcccgccgaagggctgggaagatttgactcgcattagatctccagaaaaggcccttggttacggcgggcaccgagtaaatggcg

SEQ ID NO: 2 - DNA, 2700 bp, Artificial Sequence
  misc_feature (1)..(2700): y is c or u
yggatygutauygygguuttgggutuagttuutggaguygguutygggtuygguutygggtuuutuutyggyggygtuuautgutguyguagaagagaygutuuuaggatttggtttuuagtgggagaaggaaggyguyguaaatauuatyggutgygaggygautgtggtggtygaaggaaygtgatuutttgtuagutuagyggaguygaagtgatyguygagttggutgaguagyguygagggagtttagaatuygutguagaaaauutauuaguttuttygyggauauaguaggtaatgttuttagguttutggagttagtgagtaguygguutguagguyggtaaataautuygatutaguuuuttggtttatttutttygttygyguuttgaatggaggyguuatgguauagtutgguagaggagguutguuutggygggygutautuaggguuuutgygttgagaatguygagtgaggtgutgaggtttggagagaaaaaggtggygttttuatuuuttggaatatyggguututuuagutgaaguutuyggatygauauaauauaautuuyggatygayguaauauaautuuuyguuaguuuuttuuuttuuagygggutggauauaggtgygtggguutyguaguuyggygyguayggttgyguutttggatauutgygauaggautygguuagaauygtgtuuuaggguagagaaaauuutgguaauutttaaygttutuuutgaygyggagaatuutgyguuaaygggguuttuuauttygggagautuaatyguuauuyggtuuuuaautttygtuttuuagaagaaaaatuuatgaggaggaatgggggggtuuuuygauuagauuaguaagaaaggguuuagttaggagtgauutuagyguuaygagggttuuautgutttgatgguuauayguttttguaaayggtttgggggtggagagauauuaggtgatggtagggaagggyggtggtgautgguayggutaagauautgyggagggtttygutgtggagatgagaaggtggaggttutggguautgtggutgygagtgtgagygatgygtttgtgggaatuagaggagyggatttgggaaaagtgaatuuttgagattuaggguuttautttygttaggggtgtgtgaaguauautgggtgtuaggagaggatgggaatgggattygagagguutttttttggautuutygagagaaaatggagagagtutygaauuuaggagataggaggygtattttuuuuatguauuuatggatuayguuuuyguuuuuauattuuuuuygtaggagguaagauutgagyguttautuaygtggutuuuuuatuygttuygygtuuatutuuaagautguutuauagggauuuuuaggaggutuygaauuatuuagutttutgtuauyguyguyguuauuagygttgtgaauututgauuutygyggututgygtuuattutuaggtautgaaagttttuygggututtuyguauuygyggatgtggygaaguygygggguagutuygutygygutuuagtyguaggatgtuuttgauygagaagggggtggaggtgayggggutuaguaguatuuygaaggyggatggggygggguygaggaggtuygggtgaggagygguauuutgaauttuuygtuttgtygutguagguuuyguagauagauuuaagututgggauagayguuuagygtuuuagauagyguuttuututggguuatgutggtagguuygggtuuaggguygggtgaygagauygtaguuuuuuattggttutyguagaaauuaygtgutagututguauuttuutuuuuuagygutttuttuuygyguuygtygaatuututuuagtuuuuagtyguuttuutgggaggtttggttygtattgayggttutuaaaguaaagaaaaygtggagagauagtgutgygygygguttggatutuygtuaatayggtautagygggaguttuygaggtuaauutagggtuuayggggauuutuutagtggauatgyggggattggaggtggagtuuttgutgtguaauuygatuyggtuuatuuaguutggtuttagutuaaututguattuttatggyggaggaaagutaagatagagauagutgggauuygyggaatttgaggygygygutgggatuttaygtgyguagagguyggauyguagagtagaagtgagtuttgauuuauuaggguutatattgagatggaaauututututttgaauagaatuuaggtutgyggagtuuygauuyguuauttuutaggaguaguttutuaguuuuaggauygaggaatgggtgtgggggutauatgtggggaguuutygauututtaaagggutuygygaatggtgggggagautggaagguaatututgygguuygyguaaagtggtuagaggygggagtgggggtgggggggggtggguttuygtyguuuttggygtuuuuaygttutttttuttuututuutttatuutuuttaaagyggattguutggagygtguuaguttgtgtgygygtataaatgyggyguuyguygaagggutgggaagatttgautyguattagatutuuagaaaagguuuttggttayggyggguauygagtaaatggyg

SEQ ID NO: 3 - DNA, 2700 bp, Homo sapiens
cgccatttactcggtgcccgccgtaaccaagggccttttctggagatctaatgcgagtcaaatcttcccagcccttcggcgggcgccgcatttatacgcgcacacaagctggcacgctccaggcaatccgctttaaggaggataaaggagaggaagaaaaagaacgtggggacgccaagggcgacggaagcccacccccccccacccccactcccgcctctgaccactttgcgcgggccgcagagattgccttccagtctcccccaccattcgcggagccctttaagaggtcgagggctccccacatgtagcccccacacccattcctcggtcctggggctgagaagctgctcctaggaagtggcgggtcgggactccgcagacctggattctgttcaaagagagaggtttccatctcaatataggccctggtgggtcaagactcacttctactctgcggtccggcctctgcgcacgtaagatcccagcgcgcgcctcaaattccgcgggtcccagctgtctctatcttagctttcctccgccataagaatgcagagttgagctaagaccaggctggatggaccggatcgggttgcacagcaaggactccacctccaatccccgcatgtccactaggagggtccccgtggaccctaggttgacctcggaagctcccgctagtaccgtattgacggagatccaagccgcgcgcagcactgtctctccacgttttctttgctttgagaaccgtcaatacgaaccaaacctcccaggaaggcgactggggactggagaggattcgacgggcgcgggaagaaagcgctgggggaggaaggtgcagagctagcacgtggtttctgcgagaaccaatggggggctacggtctcgtcacccggccctggacccgggcctaccagcatggcccagaggaaggcgctgtctgggacgctgggcgtctgtcccagagcttgggtctgtctgcggggcctgcagcgacaagacgggaagttcagggtgccgctcctcacccggacctcctcggccccgccccatccgccttcgggatgctgctgagccccgtcacctccacccccttctcggtcaaggacatcctgcgactggagcgcgagcggagctgccccgcggcttcgccacatccgcgggtgcggaagagcccggaaaactttcagtacctgagaatggacgcagagccgcgagggtcagaggttcacaacgctggtggcggcggcggtgacagaaagctggatggttcggagcctcctgggggtccctgtgaggcagtcttggagatggacgcggaacggatgggggagccacgtgagtaagcgctcaggtcttgcctcctacggggggaatgtgggggcgggggcgtgatccatgggtgcatggggaaaatacgcctcctatctcctgggttcgagactctctccattttctctcgaggagtccaaaaaaaggcctctcgaatcccattcccatcctctcctgacacccagtgtgcttcacacacccctaacgaaagtaaggccctgaatctcaaggattcacttttcccaaatccgctcctctgattcccacaaacgcatcgctcacactcgcagccacagtgcccagaacctccaccttctcatctccacagcgaaaccctccgcagtgtcttagccgtgccagtcaccaccgcccttccctaccatcacctggtgtctctccacccccaaaccgtttgcaaaagcgtgtggccatcaaagcagtggaaccctcgtggcgctgaggtcactcctaactgggccctttcttgctggtctggtcgggggacccccccattcctcctcatggatttttcttctggaagacgaaagttggggaccgggtggcgattgagtctcccgaagtggaaggccccgttggcgcaggattctccgcgtcagggagaacgttaaaggttgccagggttttctctgccctgggacacggttctggccgagtcctgtcgcaggtatccaaaggcgcaaccgtgcgcgccgggctgcgaggcccacgcacctgtgtccagcccgctggaagggaaggggctggcggggagttgtgttgcgtcgatccgggagttgtgttgtgtcgatccggaggcttcagctggagaggcccgatattccaagggatgaaaacgccacctttttctctccaaacctcagcacctcactcggcattctcaacgcaggggccctgagtagcgcccgccagggcaggcctcctctgccagactgtgccatggcgcctccattcaaggcgcgaacgaaagaaataaaccaaggggctagatcggagttatttaccggcctgcaggccggctactcactaactccagaagcctaagaacattacctgctgtgtccgcgaagaagctggtaggttttctgcagcggattctaaactccctcggcgctgctcagccaactcggcgatcacttcggctccgctgagctgacaaaggatcacgttccttcgaccaccacagtcgcctcgcagccgatggtatttgcggcgccttccttctcccactggaaaccaaatcctgggagcgtctcttctgcggcagcagtggacgccgccgaggagggacccgaggccggacccgaggccggctccaggaactgagcccaaggccgcggtagcgatccg

SEQ ID NO: 4 - DNA, 2700 bp, Artificial Sequence
  misc_feature (1)..(2700): y is c or u
yguuatttautyggtguuyguygtaauuaaggguuttttutggagatutaatgygagtuaaatuttuuuaguuuttyggygggyguyguatttataygyguauauaagutgguaygutuuagguaatuygutttaaggaggataaaggagaggaagaaaaagaaygtggggayguuaagggygayggaaguuuauuuuuuuuuauuuuuautuuyguututgauuautttgygyggguyguagagattguuttuuagtutuuuuuauuattygyggaguuutttaagaggtygagggutuuuuauatgtaguuuuuauauuuattuutyggtuutggggutgagaagutgutuutaggaagtggygggtygggautuyguagauutggattutgttuaaagagagaggtttuuatutuaatatagguuutggtgggtuaagautuauttutaututgyggtuygguututgyguaygtaagatuuuagygygyguutuaaattuygygggtuuuagutgtututatuttagutttuutuyguuataagaatguagagttgagutaagauuaggutggatggauyggatygggttguauaguaaggautuuauutuuaatuuuyguatgtuuautaggagggtuuuygtggauuutaggttgauutyggaagutuuygutagtauygtattgayggagatuuaaguygygyguaguautgtututuuaygttttutttgutttgagaauygtuaataygaauuaaauutuuuaggaaggygautggggautggagaggattygaygggygygggaagaaagygutgggggaggaaggtguagagutaguaygtggtttutgygagaauuaatggggggutayggtutygtuauuygguuutggauuyggguutauuaguatgguuuagaggaaggygutgtutgggaygutgggygtutgtuuuagaguttgggtutgtutgygggguutguagygauaagaygggaagttuagggtguygutuutuauuyggauutuutygguuuyguuuuatuyguuttygggatgutgutgaguuuygtuauutuuauuuuuttutyggtuaaggauatuutgygautggagygygagyggagutguuuygygguttyguuauatuygygggtgyggaagaguuyggaaaautttuagtauutgagaatggayguagaguygygagggtuagaggttuauaaygutggtggyggyggyggtgauagaaagutggatggttyggaguutuutgggggtuuutgtgagguagtuttggagatggaygyggaayggatgggggaguuaygtgagtaagygutuaggtuttguutuutayggggggaatgtgggggygggggygtgatuuatgggtguatggggaaaatayguutuutatutuutgggttygagautututuuattttututygaggagtuuaaaaaaagguututygaatuuuattuuuatuututuutgauauuuagtgtguttuauauauuuutaaygaaagtaagguuutgaatutuaaggattuauttttuuuaaatuygutuututgattuuuauaaayguatygutuauautyguaguuauagtguuuagaauutuuauuttutuatutuuauagygaaauuutuyguagtgtuttaguygtguuagtuauuauyguuuttuuutauuatuauutggtgtututuuauuuuuaaauygtttguaaaagygtgtgguuatuaaaguagtggaauuutygtggygutgaggtuautuutaautggguuutttuttgutggtutggtygggggauuuuuuuattuutuutuatggatttttuttutggaagaygaaagttggggauygggtggygattgagtutuuygaagtggaagguuuygttggyguaggattutuygygtuagggagaaygttaaaggttguuagggttttututguuutgggauayggttutgguygagtuutgtyguaggtatuuaaaggyguaauygtgygyguygggutgygagguuuayguauutgtgtuuaguuygutggaagggaaggggutggyggggagttgtgttgygtygatuygggagttgtgttgtgtygatuyggagguttuagutggagagguuygatattuuaagggatgaaaayguuauutttttututuuaaauutuaguauutuautygguattutuaayguagggguuutgagtagyguuyguuaggguagguutuututguuagautgtguuatggyguutuuattuaaggygygaaygaaagaaataaauuaaggggutagatyggagttatttauygguutguagguyggutautuautaautuuagaaguutaagaauattauutgutgtgtuygygaagaagutggtaggttttutguagyggattutaaautuuutyggygutgutuaguuaautyggygatuauttyggutuygutgagutgauaaaggatuaygttuuttygauuauuauagtyguutyguaguygatggtatttgyggyguuttuuttutuuuautggaaauuaaatuutgggagygtututtutgygguaguagtggayguyguygaggagggauuygagguyggauuygagguyggutuuaggaautgaguuuaagguygyggtagygatuyg

SEQ ID NO: 5 - DNA, 22 bp, Primer
atgaagtttatygaaggtgttt

SEQ ID NO: 6 - DNA, 24 bp, Primer
tttctctccaaacctcaacacctc

SEQ ID NO: 7 - DNA, 24 bp, Primer
gaggtgttgaggtttggagagaaa

SEQ ID NO: 8 - DNA, 24 bp, Primer
aacctccaccttctcatctccaca

SEQ ID NO: 9 - DNA, 24 bp, Primer
tgtggagatgagaaggtggaggtt

SEQ ID NO: 10 - DNA, 22 bp, Primer
atactactaaaccccrtcacct

SEQ ID NO: 11 - DNA, 22 bp, Primer
atygagaagggggtggaggtga

SEQ ID NO: 12 - DNA, 23 bp, Primer
aactaaaaccaaactaaataaac

SEQ ID NO: 13 - DNA, 23 bp, Primer
gtttatttagtttggttttagtt

SEQ ID NO: 14 - DNA, 23 bp, Primer
taataacctttataccacactac

SEQ ID NO: 15 - DNA, 25 bp, Primer
gaggygattgtggtggtygaaggaa

SEQ ID NO: 16 - DNA, 29 bp, Primer
aaactccctcracrctactcaaccaactc

SEQ ID NO: 17 - DNA, 28 bp, Primer
gaaggaaygtgattttttgttagtttag

SEQ ID NO: 18 - DNA, 40 bp, Primer
yggagtygaagtgatygtygagttggttgagtagygtyga